European Patent Application EP 4 289 862 A1, published December 13, 2023. Title: ANTI-HUMAN B7-H3 ANTIBODY AND APPLICATION THEREOF. Applicant: MABWELL (SHANGHAI) BIOSCIENCE CO., LTD. The sequence listing filed with the application follows.

SEQUENCE LISTING (60 sequences)

SEQ ID NO: 1 - protein, 122 aa, Artificial Sequence
EVQLQQSGPELVRPGVSVKISCKGSGYSFTDYAIHWVKQSHAMSLEWIGIINTYYGNTNYNQKFKGKATMTVDKSSSTAYMELARLTSADSAIYYCARSTTTATFYWYFDVWGAGTTVSVSS

SEQ ID NO: 2 - protein, 107 aa, Artificial Sequence
DIVLTQSPVTLSVTPGDSVSLSCRASQSINNNLHWYQQKPHESPRLLIKYASQSISGIPSRFSGSGSGTDFTLSFNSVETEDFGMYFCQQSHSWPYTFGGGTKLEIK

SEQ ID NO: 3 - protein, 121 aa, Artificial Sequence
EVQLQQSGPELVKPGASVKISCKTSGYTFTEYIMHWVKQSHGKSLEWIGGINPNNGGTTYNQKFKGKATLTVDKSSSTAYMELRSLTSEDSAVYYCARKGKDYFDWYFDVWGAGTTVTVSS

SEQ ID NO: 4 - protein, 106 aa, Artificial Sequence
QIVLTQSPTIMSASPGEKVTMTCSASSSVSYMHWYQQKSGTSPKRWIYDTSKLASGVPARFSGSGSGTSYSLTISSMEAEDAATYYCQQWSSNPLTFGAGTKLELK

SEQ ID NO: 5 - protein, 124 aa, Artificial Sequence
QVQLQQSGPELVRPGVSVKISCKGSGYTFTDYALHWVKQSHAKSPQWIGLINTYSSNTNYNQKFKDKATMTVDKSSSTAYMELARLTSEDSAIYYCARGITAVVGTRYYAMDYWGQGTSVTVSS

SEQ ID NO: 6 - protein, 113 aa, Artificial Sequence
NIVLTQSPTTLSVTPGDTVSLSCRASQSISNNLHWYQQRSHESPRLIIKYTSQNISGIPSRFSGSGSGTDFTLSINSVETEDFGMYFCQQSYSWPLTFGAGTKLELKRADAAP

SEQ ID NO: 7 - protein, 452 aa, Artificial Sequence
EVQLVESGGGLVQPGGSLRLSCAASGFTFSSFGMHWVRQAPGKGLEWVAYISSDSSAIYYADTVKGRFTISRDNAKNSLYLQMNSLRDEDTAVYYCGRGRENIYYGSRLDYWGQGTTVTVSSASTKGPSVFPLAPSSKSTSGGTAALGCLVKDYFPEPVTVSWNSGALTSGVHTFPAVLQSSGLYSLSSVVTVPSSSLGTQTYICNVNHKPSNTKVDKRVEPKSCDKTHTCPPCPAPELVGGPSVFLLPPKPKDTLMISRTPEVTCVVVDVSHEDPEVKFNWYVDGVEVHNAKTKPPEEQYNSTLRVVSVLTVLHQDWLNGKEYKCKVSNKALPAPIEKTISKAKGQPREPQVYTLPPSREEMTKNQVSLTCLVKGFYPSDIAVEWESNGQPENNYKTTPLVLDSDGSFFLYSKLTVDKSRWQQGNVFSCSVMHEALHNHYTQKSLSLSPGK

SEQ ID NO: 8 - protein, 214 aa, Artificial Sequence
DIQLTQSPSFLSASVGDRVTITCKASQNVDTNVAWYQQKPGKAPKALIYSASYRYSGVPSRFSGSGSGTDFTLTISSLQPEDFATYYCQQYNNYPFTFGQGTKLEIKRTVAAPSVFIFPPSDEQLKSGTASVVCLLNNFYPREAKVQWKVDNALQSGNSQESVTEQDSKDSTYSLSSTLTLSKADYEKHKVYACEVTHQGLSSPVTKSFNRGEC

SEQ ID NO: 9 - protein, 447 aa, Artificial Sequence
EVQLVESGGGLVKPGGSLRLSCAASGFTFSSYGMSWVRQAPGKGLEWVATINSGGSNTYYPDSLKGRFTISRDNAKNSLYLQMNSLRAEDTAVYYCARHDGGAMDYWGQGTTVTVSSASTKGPSVFPLAPSSKSTSGGTAALGCLVKDYFPEPVTVSWNSGALTSGVHTFPAVLQSSGLYSLSSVVTVPSSSLGTQTYICNVNHKPSNTKVDKRVEPKSCDKTHTCPPCPAPELLGGPSVFLFPPKPKDTLMISRTPEVTCVVVDVSHEDPEVKFNWYVDGVEVHNAKTKPREEQYNSTYRVVSVLTVLHQDWLNGKEYKCKVSNKALPAPIEKTISKAKGQPREPQVYTLPPSREEMTKNQVSLTCLVKGFYPSDIAVEWESNGQPENNYKTTPPVLDSDGSFFLYSKLTVDKSRWQQGNVFSCSVMHEALHNHYTQKSLSLSPGK

SEQ ID NO: 10 - protein, 215 aa, Artificial Sequence
DIQMTQSPSSLSASVGDRVTITCRASESIYSYLAWYQQKPGKAPKLLVYNTKTLPEGVPSRFSGSGSGTDFTLTISSLQPEDFATYYCQHHYGTPPWTFGQGTRLEIKRTVAAPSVFIFPPSDEQLKSGTASVVCLLNNFYPREAKVQWKVDNALQSGNSQESVTEQDSKDSTYSLSSTLTLSKADYEKHKVYACEVTHQGLSSPVTKSFNRGEC

SEQ ID NO: 11 - protein, 122 aa, Artificial Sequence
QVQLVQSGAEVKKPGASVKVSCKASGYTFTDYAIHWVRQAPGQGLEWMGIINTYYGNTNYNQKFKGRVTMTRDTSISTAYMELSRLRSDDTAVYYCARSTTTATFYWYFDVWGQGTTVTVSS

SEQ ID NO: 12 - protein, 107 aa, Artificial Sequence
EIVLTQSPGTLSLSPGERATLSCRASQSINNNLHWYQQKPGQAPRLLIYYASQSISGIPDRFSGSGSGTDFTLTISRLEPEDFAVYYCQQSHSWPYTFGQGTKLEIK

SEQ ID NO: 13 - protein, 107 aa, Artificial Sequence
EIVLTQSPDFQSVTPKEKVTITCRASQSINNNLHWYQQKPDQSPKLLIKYASQSISGVPSRFSGSGSGTDFTLTINSLEAEDAATYYCQQSHSWPYTFGQGTKLEIK

SEQ ID NO: 14 - protein, 107 aa, Artificial Sequence
EIVLTQSPGTLSLSPGERATLSCRASQSINNNLHWYQQKPGQAPRLLIKYASQSISGIPDRFSGSGSGTDFTLTISRLEPEDFAVYYCQQSHSWPYTFGQGTKLEIK

SEQ ID NO: 15 - protein, 107 aa, Artificial Sequence
EIVLTQSPGTLSLSPGERATLSCRASQSINNNLHWYQQKPGQAPRLLIYYASQSISGIPDRFSGSGSGTDFTLTISRLEPEDFAVYFCQQSHSWPYTFGQGTKLEIK

SEQ ID NO: 16 - protein, 107 aa, Artificial Sequence
EIVLTQSPGTLSLSPGERATLSCRASQSINNNLHWYQQKPGQAPRLLIKYASQSISGIPDRFSGSGSGTDFTLTISRLEPEDFAVYFCQQSHSWPYTFGQGTKLEIK

SEQ ID NO: 17 - protein, 122 aa, Artificial Sequence
EVQLVQSGAEVKKPGASVKVSCKASGYTFTDYAIHWVRQAPGQGLEWMGIINTYYGNTNYNQKFKGRVTMTRDTSISTAYMELSRLRSDDTAVYYCARSTTTATFYWYFDVWGQGTTVTVSS

SEQ ID NO: 18 - protein, 121 aa, Artificial Sequence
QVQLVQSGAEVKKPGASVKVSCKASGYTFTEYIMHWVRQAPGQGLEWMGGINPNNGGTTYNQKFKGRVTMTRDTSISTAYMELSRLRSDDTAVYYCARKGKDYFDWYFDVWGQGTTVTVSS

SEQ ID NO: 19 - protein, 106 aa, Artificial Sequence
DIQMTQSPSSLSASVGDRVTMTCSASSSVSYMHWYQQKPGKAPKLLIYDTSKLASGVPSRFSGSGSGTDFTLTISSLQPEDFATYYCQQWSSNPLTFGGGTKVEIK

SEQ ID NO: 20 - protein, 106 aa, Artificial Sequence
DIQLTQSPSSLSASVGDRVTMTCSASSSVSYMHWYQQKPGKAPKLLIYDTSKLASGVPSRFSGSGSGTDFTLTISSLQPEDFATYYCQQWSSNPLTFGGGTKVEIK

SEQ ID NO: 21 - protein, 121 aa, Artificial Sequence
EVQLVQSGAEVKKPGASVKVSCKASGYTFTEYIMHWVRQAPGQGLEWMGGINPNNGGTTYNQKFKGRVTMTRDTSISTAYMELSRLRSEDTAVYYCARKGKDYFDWYFDVWGQGTTVTVSS

SEQ ID NO: 22 - protein, 121 aa, Artificial Sequence
EVQLVQSGAEVKKPGASVKVSCKASGYTFTEYIMHWVRQAPGQGLEWMGGINPASGGTTYNQKFKGRVTMTRDTSISTAYMELSRLRSEDTAVYYCARKGKDYFDWYFDVWGQGTTVTVSS

SEQ ID NO: 23 - protein, 121 aa, Artificial Sequence
EVQLVQSGAEVKKPGASVKVSCKASGYTFTEYIMHWVRQAPGQGLEWMGGINPNQGGTTYNQKFKGRVTMTRDTSISTAYMELSRLRSEDTAVYYCARKGKDYFDWYFDVWGQGTTVTVSS

SEQ ID NO: 24 - protein, 124 aa, Artificial Sequence
QVQLVQSGAEVKKPGASVKVSCKASGYTFTDYALHWVRQAPGQGLEWMGLINTYSSNTNYNQKFKDRVTMTRDTSISTAYMELSRLRSDDTAVYYCARGITAVVGTRYYAMDYWGQGTLVTVSS

SEQ ID NO: 25 - protein, 107 aa, Artificial Sequence
EIVLTQSPGTLSLSPGERATLSCRASQSISNNLHWYQQKPGQAPRLLIYYTSQNISGIPDRFSGSGSGTDFTLTISRLEPEDFAVYYCQQSYSWPLTFGGGTKVEIK

SEQ ID NO: 26 - protein, 107 aa, Artificial Sequence
EIVLTQSPDFQSVTPKEKVTITCRASQSISNNLHWYQQKPDQSPKLLIYYTSQNISGVPSRFSGSGSGTDFTLTINSLEAEDAATYYCQQSYSWPLTFGGGTKVEIK

SEQ ID NO: 27 - protein, 107 aa, Artificial Sequence
EIVLTQSPGTLSLSPGERATLSCRASQSISNNLHWYQQKPGQAPRLLIKYTSQNISGIPDRFSGSGSGTDFTLTISRLEPEDFAVYYCQQSYSWPLTFGGGTKVEIK

SEQ ID NO: 28 - protein, 107 aa, Artificial Sequence
EIVLTQSPGTLSLSPGERATLSCRASQSISNNLHWYQQKPGQAPRLLIYYTSQNISGIPDRFSGSGSGTDFTLTISRLEPEDFAVYFCQQSYSWPLTFGGGTKVEIK

SEQ ID NO: 29 - protein, 107 aa, Artificial Sequence
EIVLTQSPGTLSLSPGERATLSCRASQSISSNLHWYQQKPGQAPRLLIKYTSQNISGIPDRFSGSGSGTDFTLTISRLEPEDFAVYYCQQSYSWPLTFGGGTKVEIK

SEQ ID NO: 30 - protein, 107 aa, Artificial Sequence
EIVLTQSPGTLSLSPGERATLSCRASQSISNNLHWYQQKPGQAPRLLIKYTSQSISGIPDRFSGSGSGTDFTLTISRLEPEDFAVYYCQQSYSWPLTFGGGTKVEIK

SEQ ID NO: 31 - protein, 107 aa, Artificial Sequence
EIVLTQSPGTLSLSPGERATLSCRASQSISSNLHWYQQKPGQAPRLLIKYTSQSISGIPDRFSGSGSGTDFTLTISRLEPEDFAVYYCQQSYSWPLTFGGGTKVEIK

SEQ ID NO: 32 - protein, 107 aa, Artificial Sequence
EIVLTQSPDFQSVTPKEKVTITCRASQSISNNLHWYQQKPDQSPKLLIKYTSQNISGVPSRFSGSGSGTDFTLTINSLEAEDAATYYCQQSYSWPLTFGGGTKVEIK

SEQ ID NO: 33 - protein, 107 aa, Artificial Sequence
EIVLTQSPDFQSVTPKEKVTITCRASQSISNNLHWYQQKPDQSPKLLIYYTSQNISGVPSRFSGSGSGTDFTLTINSLEAEDAATYFCQQSYSWPLTFGGGTKVEIK

SEQ ID NO: 34 - protein, 124 aa, Artificial Sequence
QVQLVQSGAEVKKPGASVKVSCKASGYTFTDYALHWVRQAPGQGLEWIGLINTYSSNTNYNQKFKDRVTMTRDTSISTAYMELSRLRSDDTAVYYCARGITAVVGTRYYAMDYWGQGTLVTVSS

SEQ ID NO: 35 - protein, 124 aa, Artificial Sequence
EVQLVQSGAEVKKPGASVKVSCKASGYTFTDYALHWVRQAPGQGLEWMGLINTYSSNTNYNQKFKDRVTMTRDTSISTAYMELSRLRSEDTAVYYCARGITAVVGTRYYAMDYWGQGTLVTVSS

SEQ ID NO: 36 - protein, 124 aa, Artificial Sequence
EVQLVQSGAEVKKPGASVKVSCKASGYTFTDYALHWVRQAPGQGLEWMGLISTYSSNTNYNQKFKDRVTMTRDTSISTAYMELSRLRSEDTAVYYCARGITAVVGTRYYAMDYWGQGTLVTVSS

SEQ ID NO: 37 - protein, 124 aa, Artificial Sequence
EVQLVQSGAEVKKPGASVKVSCKASGYTFTDYALHWVRQAPGQGLEWMGLINTYSSSTNYNQKFKDRVTMTRDTSISTAYMELSRLRSEDTAVYYCARGITAVVGTRYYAMDYWGQGTLVTVSS

SEQ ID NO: 38 - protein, 330 aa, Artificial Sequence
ASTKGPSVFPLAPSSKSTSGGTAALGCLVKDYFPEPVTVSWNSGALTSGVHTFPAVLQSSGLYSLSSVVTVPSSSLGTQTYICNVNHKPSNTKVDKRVEPKSCDKTHTCPPCPAPELLGGPSVFLFPPKPKDTLMISRTPEVTCVVVDVSHEDPEVKFNWYVDGVEVHNAKTKPREEQYNSTYRVVSVLTVLHQDWLNGKEYKCKVSNKALPAPIEKTISKAKGQPREPQVYTLPPSREEMTKNQVSLTCLVKGFYPSDIAVEWESNGQPENNYKTTPPVLDSDGSFFLYSKLTVDKSRWQQGNVFSCSVMHEALHNHYTQKSLSLSPGK

SEQ ID NO: 39 - protein, 107 aa, Artificial Sequence [sequence omitted]

SEQ ID NO: 40 - protein, 5 aa, Artificial Sequence
DYAIH

SEQ ID NO: 41 - protein, 17 aa, Artificial Sequence
IINTYYGNTNYNQKFKG

SEQ ID NO: 42 - protein, 13 aa, Artificial Sequence
STTTATFYWYFDV

SEQ ID NO: 43 - protein, 11 aa, Artificial Sequence
RASQSINNNLH

SEQ ID NO: 44 - protein, 7 aa, Artificial Sequence
YASQSIS

SEQ ID NO: 45 - protein, 9 aa, Artificial Sequence
QQSHSWPYT

SEQ ID NO: 46 - protein, 5 aa, Artificial Sequence
EYIMH

SEQ ID NO: 47 - protein, 17 aa, Artificial Sequence
GINPNNGGTTYNQKFKG

SEQ ID NO: 48 - protein, 12 aa, Artificial Sequence
KGKDYFDWYFDV

SEQ ID NO: 49 - protein, 10 aa, Artificial Sequence
SASSSVSYMH

SEQ ID NO: 50 - protein, 7 aa, Artificial Sequence
DTSKLAS

SEQ ID NO: 51 - protein, 9 aa, Artificial Sequence
QQWSSNPLT

SEQ ID NO: 52 - protein, 5 aa, Artificial Sequence
DYALH

SEQ ID NO: 53 - protein, 17 aa, Artificial Sequence
LINTYSSNTNYNQKFKD

SEQ ID NO: 54 - protein, 15 aa, Artificial Sequence
GITAVVGTRYYAMDY

SEQ ID NO: 55 - protein, 11 aa, Artificial Sequence
RASQSISNNLH

SEQ ID NO: 56 - protein, 7 aa, Artificial Sequence
YTSQNIS

SEQ ID NO: 57 - protein, 9 aa, Artificial Sequence
QQSYSWPLT

SEQ ID NO: 58 - protein, 106 aa, Artificial Sequence
DIQLTQSPSSLSASVGDRVTMTCSASSSVSYMHWYQQKPGKAPKLLIYDTSKLASGVPSRFSGSGSGTDFTLTISSLQPEDFATYYCQQWSSAPLTFGGGTKVEIK

SEQ ID NO: 59 - protein, 106 aa, Artificial Sequence
DIQLTQSPSSLSASVGDRVTMTCSASSSVSYMHWYQQKPGKAPKLLIYDTSKLASGVPSRFSGSGSGTDFTLTISSLQPEDFATYYCQQWSASPLTFGGGTKVEIK

SEQ ID NO: 60 - protein, 106 aa, Artificial Sequence
DIQLTQSPSSLSASVGDRVTMTCSASSSVSYMHWYQQKPGKAPKLLIYDTSKLASGVPSRFSGSGSGTDFTLTISSLQPEDFATYYCQQWSSQPLTFGGGTKVEIK